European Patent Application EP 4 389 760 A1, published June 26, 2024. Title: ISOLATED MODIFIED AAV9 CAPSID PROTEIN VP1. Applicant: Joint Stock Company «BIOCAD». Application WO PCT/RU2022/050258, filed August 21, 2022. The sequence listing filed with the application follows.

SEQUENCE LISTING (24 sequences)

SEQ ID NO: 1 - protein, 736 aa, Adeno-associated dependoparvovirus A
MAADGYLPDWLEDNLSEGIREWWALKPGAPQPKANQQHQDNARGLVLPGYKYLGPGNGLDKGEPVNAADAAALEHDKAYDQQLKAGDNPYLKYNHADAEFQERLKEDTSFGGNLGRAVFQAKKRLLEPLGLVEEAAKTAPGKKRPVEQSPQEPDSSAGIGKSGAQPAKKRLNFGQTGDTESVPDPQPIGEPPAAPSGVGSLTMASGGGAPVADNNEGADGVGSSSGNWHCDSQWLGDRVITTSTRTWALPTYNNHLYKQISNSTSGGSSNDNAYFGYSTPWGYFDFNRFHCHFSPRDWQRLINNNWGFRPKRLNFKLFNIQVKEVTDNNGVKTIANNLTSTVQVFTDSDYQLPYVLGSAHEGCLPPFPADVFMIPQYGYLTLNDGSQAVGRSSFYCLEYFPSQMLRTGNNFQFSYEFENVPFHSSYAHSQSLDRLMNPLIDQYLYYLSKTINGSGQNQQTLKFSVAGPSNMAVQGRNYIPGPSYRQQRVSTTVTQNNNSEFAWPGASSWALNGRNSLMNPGPAMASHKEGEDRFFPLSGSLIFGKQGTGRDNVDADKVMITNEEEIKTTNPVATESYGQVATNHQSAQAQAQTGWVQNQGILPGMVWQDRDVYLQGPIWAKIPHTDGNFHPSPLMGGFGMKHPPPQILIKNTPVPADPPTAFNKDKLNSFITQYSTGQVSVEIEWELQKENSKRWNPEIQYTSNYYKSNNVEFAVNTEGVYSEPRPIGTRYLTRNL

SEQ ID NO: 2 - protein, 736 aa, synthetic construct
MAADGYLPDWLEDNLSEGIREWWALKPGAPQPKANQQHQDNARGLVLPGYKYLGPGNGLDKGEPVNAADAAALEHDKAYDQQLKAGDNPYLKYNHADAEFQERLKEDTSFGGNLGRAVFQAKKRLLEPLGLVEEAAKTAPGKKRPVEQSPQEPDSSAGIGKSGAQPAKKRLNFGQTGDTESVPDPQPIGEPPAAPSGVGSLTMASGGGAPVADNNEGADGVGSSSGNWHCDSQWLGDRVITTSTRTWALPTYNNHLYKQISNSTSGGSSNDNAYFGYSTPWGYFDFNRFHCHFSPRDWQRLINNNWGFRPKRLNFKLFNIQVKEVTDNNGVKTIANNLTSTVQVFTDSDYQLPYVLGSAHEGCLPPFPADVFMIPQYGYLTLNDGSQAVGRSSFYCLEYFPSQMLRTGNNFQFSYEFENVPWHSSYAHSQSLDRLMNPLIDQYLYYLSKTINGSGQNQQTLKFSVAGPSNMAVQGRNYIPGPSYRQQRVSTTVTQNNNSEFAWPGASSWALNGRNSLMNPGPAMASHKEGEDRFFPLSGSLIFGKQGTGRDNVDADKVMITNEEEIKTTNPVATESYGQVATNHQSAQAQAQTGWVQNQGILPGMVWQDRDVYLQGPIWAKIPHTDGNFHPSPLMGGFGMKHPPPQILIKNTPVPADPPTAFNKDKLNSFITQYSTGQVSVEIEWELQKENSKRWNPEIQYTSNYYKSNNVEFAVNTEGVYSEPRPIGTRYLTRNL

SEQ ID NO: 3 - protein, 736 aa, synthetic construct
MAADGYLPDWLEDNLSEGIREWWALKPGAPQPKANQQHQDNARGLVLPGYKYLGPGNGLDKGEPVNAADAAALEHDKAYDQQLKAGDNPYLKYNHADAEFQERLKEDTSFGGNLGRAVFQAKKRLLEPLGLVEEAAKTAPGKKRPVEQSPQEPDSSAGIGKSGAQPAKKRLNFGQTGDTESVPDPQPIGEPPAAPSGVGSLTMASGGGAPVADNNEGADGVGSSSGNWHCDSQWLGDRVITTSTRTWALPTYNNHLYKQISNSTSGGSSNDNAYFGYSTPWGYFDFNRFHCHFSPRDWQRLINNNWGFRPKRLNFKLFNIQVKEVTDNNGVKTIANNLTSTVQVFTDSDYQLPYVLGSAHEGCLPPFPADVFMIPQYGYLTLNDGSQAVGRSSFYCLEYFPSQMLRTGNNFQFSYEFENVPWHSSYAHSQSLDRLMNPLIDQYLYFLSKTINGSGQNQQTLKFSVAGPSNMAVQGRNYIPGPSYRQQRVSTTVTQNNNSEFAWPGASSWALNGRNSLMNPGPAMASHKEGEDRFFPLSGSLIFGKQGTGRDNVDADKVMITNEEEIKTTNPVATESYGQVATNHQSAQAQAQTGWVQNQGILPGMVWQDRDVYLQGPIWAKIPHTDGNFHPSPLMGGFGMKHPPPQILIKNTPVPADPPTAFNKDKLNSFITQYSTGQVSVEIEWELQKENSKRWNPEIQYTSNYYKSNNVEFAVNTEGVYSEPRPIGTRYLTRNL

SEQ ID NO: 4 - protein, 736 aa, synthetic construct
MAADGYLPDWLEDNLSEGIREWWALKPGAPQPKANQQHQDNARGLVLPGYKYLGPGNGLDKGEPVNAADAAALEHDKAYDQQLKAGDNPYLKYNHADAEFQERLKEDTSFGGNLGRAVFQAKKRLLEPLGLVEEAAKTAPGKKRPVEQSPQEPDSSAGIGKSGAQPAKKRLNFGQTGDTESVPDPQPIGEPPAAPSGVGSLTMASGGGAPVADNNEGADGVGSSSGNWHCDSQWLGDRVITTSTRTWALPTYNNHLYKQISNSTSGGSSNDNAYFGYSTPWGYFDFNRFHCHFSPRDWQRLINNNWGFRPKRLNFKLFNIQVKEVTDNNGVKTIANNLTSTVQVFTDSDYQLPYVLGSAHEGCLPPFPADVFMIPQYGYLTLNDGSQAVGRSSFYCLEYFPSQMLRTGNNFQFSYEFENVPFHSSYAHSQSLDRLMNPLIDQYLYYLSKTINGSGQNQQTLKFSVAGPSNMAVQGRNYIPGPSYRQQRVSTTVTQNNNSEFAWPGASSWALNGRNSLMNPGPAMASHKEGEDRFFPLSGSLIFGKQGTGRDNVDADKVMITNEEEIKTTNPVATESYGQVATNHQSAQAQAQTGWVQNQGMLPGMVWQDRDVYLQGPIWAKIPHTDGNFHPSPLMGGFGMKHPPPQILIKNTPVPADPPTAFNKDKLNSFITQYSTGQVSVEIEWELQKENSKRWNPEIQYTSNYYKSNNVEFAVNTEGVYSEPRPIGTRYLTRNL

SEQ ID NO: 5 - DNA, 2211 bp, Adeno-associated dependoparvovirus A
  source 1..2211: mol_type = genomic DNA
atggctgccgatggttatcttccagattggctcgaggacaaccttagtgaaggaattcgcgagtggtgggctttgaaacctggagcccctcaacccaaggcaaatcaacaacatcaagacaacgctcgaggtcttgtgcttccgggttacaaataccttggacccggcaacggactcgacaagggggagccggtcaacgcagcagacgcggcggccctcgagcacgacaaggcctacgaccagcagctcaaggccggagacaacccgtacctcaagtacaaccacgccgacgccgagttccaggagcggctcaaagaagatacgtcttttgggggcaacctcgggcgagcagtcttccaggccaaaaagaggcttcttgaacctcttggtctggttgaggaagcggctaagacggctcctggaaagaagaggcctgtagagcagtctcctcaggaaccggactcctccgcgggtattggcaaatcgggtgcacagcccgctaaaaagagactcaatttcggtcagactggcgacacagagtcagtcccagaccctcaaccaatcggagaacctcccgcagccccctcaggtgtgggatctcttacaatggcttcaggtggtggcgcaccagtggcagacaataacgaaggtgccgatggagtgggtagttcctcgggaaattggcattgcgattcccaatggctgggggacagagtcatcaccaccagcacccgaacctgggccctgcccacctacaacaatcacctctacaagcaaatctccaacagcacatctggaggatcttcaaatgacaacgcctacttcggctacagcaccccctgggggtattttgacttcaacagattccactgccacttctcaccacgtgactggcagcgactcatcaacaacaactggggattccggcctaagcgactcaacttcaagctcttcaacattcaggtcaaagaggttacggacaacaatggagtcaagaccatcgccaataaccttaccagcacggtccaggtcttcacggactcagactatcagctcccgtacgtgctcgggtcggctcacgagggctgcctcccgccgttcccagcggacgttttcatgattcctcagtacgggtatctgacgcttaatgatggaagccaggccgtgggtcgttcgtccttttactgcctggaatatttcccgtcgcaaatgctaagaacgggtaacaacttccagttcagctacgagtttgagaacgtacctttccatagcagctacgctcacagccaaagcctggaccgactaatgaatccactcatcgaccaatacttgtactatctctcaaagactattaacggttctggacagaatcaacaaacgctaaaattcagtgtggccggacccagcaacatggctgtccagggaagaaactacatacctggacccagctaccgacaacaacgtgtctcaaccactgtgactcaaaacaacaacagcgaatttgcttggcctggagcttcttcttgggctctcaatggacgtaatagcttgatgaatcctggacctgctatggccagccacaaagaaggagaggaccgtttctttcctttgtctggatctttaatttttggcaaacaaggaactggaagagacaacgtggatgcggacaaagtcatgataaccaacgaagaagaaattaaaactactaacccggtagcaacggagtcctatggacaagtggccacaaaccaccagagtgcccaagcacaggcgcagaccggctgggttcaaaaccaaggaatacttccgggtatggtttggcaggacagagatgtgtacctgcaaggacccatttgggccaaaattcctcacacggacggcaactttcacccttctccgctgatgggagggtttggaatgaagcacccgcctcctcagatcctcatcaaaaacacacctgtacctgcggatcctccaacggccttcaacaaggacaagctgaactctttcatcacccagtattctactggccaagtcagcgtggagatcgagtgggagctgcagaaggaaaacagcaagcgctggaacccggagatccagtacacttccaactattacaagtctaataatgttgaatttgctgttaatactgaaggtgtatatagtgaaccccgccccattggcaccagatacctgactcgtaatctgtaa

SEQ ID NO: 6 - DNA, 2211 bp, synthetic construct
  source 1..2211: mol_type = other DNA
atggctgccgatggttatcttccagattggctcgaggacaaccttagtgaaggaattcgcgagtggtgggctttgaaacctggagcccctcaacccaaggcaaatcaacaacatcaagacaacgctcgaggtcttgtgcttccgggttacaaataccttggacccggcaacggactcgacaagggggagccggtcaacgcagcagacgcggcggccctcgagcacgacaaggcctacgaccagcagctcaaggccggagacaacccgtacctcaagtacaaccacgccgacgccgagttccaggagcggctcaaagaagatacgtcttttgggggcaacctcgggcgagcagtcttccaggccaaaaagaggcttcttgaacctcttggtctggttgaggaagcggctaagacggctcctggaaagaagaggcctgtagagcagtctcctcaggaaccggactcctccgcgggtattggcaaatcgggtgcacagcccgctaaaaagagactcaatttcggtcagactggcgacacagagtcagtcccagaccctcaaccaatcggagaacctcccgcagccccctcaggtgtgggatctcttacaatggcttcaggtggtggcgcaccagtggcagacaataacgaaggtgccgatggagtgggtagttcctcgggaaattggcattgcgattcccaatggctgggggacagagtcatcaccaccagcacccgaacctgggccctgcccacctacaacaatcacctctacaagcaaatctccaacagcacatctggaggatcttcaaatgacaacgcctacttcggctacagcaccccctgggggtattttgacttcaacagattccactgccacttctcaccacgtgactggcagcgactcatcaacaacaactggggattccggcctaagcgactcaacttcaagctcttcaacattcaggtcaaagaggttacggacaacaatggagtcaagaccatcgccaataaccttaccagcacggtccaggtcttcacggactcagactatcagctcccgtacgtgctcgggtcggctcacgagggctgcctcccgccgttcccagcggacgttttcatgattcctcagtacgggtatctgacgcttaatgatggaagccaggccgtgggtcgttcgtccttttactgcctggaatatttcccgtcgcaaatgctaagaacgggtaacaacttccagttcagctacgagtttgagaacgtaccttggcatagcagctacgctcacagccaaagcctggaccgactaatgaatccactcatcgaccaatacttgtactatctctcaaagactattaacggttctggacagaatcaacaaacgctaaaattcagtgtggccggacccagcaacatggctgtccagggaagaaactacatacctggacccagctaccgacaacaacgtgtctcaaccactgtgactcaaaacaacaacagcgaatttgcttggcctggagcttcttcttgggctctcaatggacgtaatagcttgatgaatcctggacctgctatggccagccacaaagaaggagaggaccgtttctttcctttgtctggatctttaatttttggcaaacaaggaactggaagagacaacgtggatgcggacaaagtcatgataaccaacgaagaagaaattaaaactactaacccggtagcaacggagtcctatggacaagtggccacaaaccaccagagtgcccaagcacaggcgcagaccggctgggttcaaaaccaaggaatacttccgggtatggtttggcaggacagagatgtgtacctgcaaggacccatttgggccaaaattcctcacacggacggcaactttcacccttctccgctgatgggagggtttggaatgaagcacccgcctcctcagatcctcatcaaaaacacacctgtacctgcggatcctccaacggccttcaacaaggacaagctgaactctttcatcacccagtattctactggccaagtcagcgtggagatcgagtgggagctgcagaaggaaaacagcaagcgctggaacccggagatccagtacacttccaactattacaagtctaataatgttgaatttgctgttaatactgaaggtgtatatagtgaaccccgccccattggcaccagatacctgactcgtaatctgtaa

SEQ ID NO: 7 - DNA, 2211 bp, synthetic construct
  source 1..2211: mol_type = other DNA
atggctgccgatggttatcttccagattggctcgaggacaaccttagtgaaggaattcgcgagtggtgggctttgaaacctggagcccctcaacccaaggcaaatcaacaacatcaagacaacgctcgaggtcttgtgcttccgggttacaaataccttggacccggcaacggactcgacaagggggagccggtcaacgcagcagacgcggcggccctcgagcacgacaaggcctacgaccagcagctcaaggccggagacaacccgtacctcaagtacaaccacgccgacgccgagttccaggagcggctcaaagaagatacgtcttttgggggcaacctcgggcgagcagtcttccaggccaaaaagaggcttcttgaacctcttggtctggttgaggaagcggctaagacggctcctggaaagaagaggcctgtagagcagtctcctcaggaaccggactcctccgcgggtattggcaaatcgggtgcacagcccgctaaaaagagactcaatttcggtcagactggcgacacagagtcagtcccagaccctcaaccaatcggagaacctcccgcagccccctcaggtgtgggatctcttacaatggcttcaggtggtggcgcaccagtggcagacaataacgaaggtgccgatggagtgggtagttcctcgggaaattggcattgcgattcccaatggctgggggacagagtcatcaccaccagcacccgaacctgggccctgcccacctacaacaatcacctctacaagcaaatctccaacagcacatctggaggatcttcaaatgacaacgcctacttcggctacagcaccccctgggggtattttgacttcaacagattccactgccacttctcaccacgtgactggcagcgactcatcaacaacaactggggattccggcctaagcgactcaacttcaagctcttcaacattcaggtcaaagaggttacggacaacaatggagtcaagaccatcgccaataaccttaccagcacggtccaggtcttcacggactcagactatcagctcccgtacgtgctcgggtcggctcacgagggctgcctcccgccgttcccagcggacgttttcatgattcctcagtacgggtatctgacgcttaatgatggaagccaggccgtgggtcgttcgtccttttactgcctggaatatttcccgtcgcaaatgctaagaacgggtaacaacttccagttcagctacgagtttgagaacgtaccttggcatagcagctacgctcacagccaaagcctggaccgactaatgaatccactcatcgaccaatacttgtactttctctcaaagactattaacggttctggacagaatcaacaaacgctaaaattcagtgtggccggacccagcaacatggctgtccagggaagaaactacatacctggacccagctaccgacaacaacgtgtctcaaccactgtgactcaaaacaacaacagcgaatttgcttggcctggagcttcttcttgggctctcaatggacgtaatagcttgatgaatcctggacctgctatggccagccacaaagaaggagaggaccgtttctttcctttgtctggatctttaatttttggcaaacaaggaactggaagagacaacgtggatgcggacaaagtcatgataaccaacgaagaagaaattaaaactactaacccggtagcaacggagtcctatggacaagtggccacaaaccaccagagtgcccaagcacaggcgcagaccggctgggttcaaaaccaaggaatacttccgggtatggtttggcaggacagagatgtgtacctgcaaggacccatttgggccaaaattcctcacacggacggcaactttcacccttctccgctgatgggagggtttggaatgaagcacccgcctcctcagatcctcatcaaaaacacacctgtacctgcggatcctccaacggccttcaacaaggacaagctgaactctttcatcacccagtattctactggccaagtcagcgtggagatcgagtgggagctgcagaaggaaaacagcaagcgctggaacccggagatccagtacacttccaactattacaagtctaataatgttgaatttgctgttaatactgaaggtgtatatagtgaaccccgccccattggcaccagatacctgactcgtaatctgtaa

SEQ ID NO: 8 - DNA, 2211 bp, synthetic construct
  source 1..2211: mol_type = other DNA
atggctgccgatggttatcttccagattggctcgaggacaaccttagtgaaggaattcgcgagtggtgggctttgaaacctggagcccctcaacccaaggcaaatcaacaacatcaagacaacgctcgaggtcttgtgcttccgggttacaaataccttggacccggcaacggactcgacaagggggagccggtcaacgcagcagacgcggcggccctcgagcacgacaaggcctacgaccagcagctcaaggccggagacaacccgtacctcaagtacaaccacgccgacgccgagttccaggagcggctcaaagaagatacgtcttttgggggcaacctcgggcgagcagtcttccaggccaaaaagaggcttcttgaacctcttggtctggttgaggaagcggctaagacggctcctggaaagaagaggcctgtagagcagtctcctcaggaaccggactcctccgcgggtattggcaaatcgggtgcacagcccgctaaaaagagactcaatttcggtcagactggcgacacagagtcagtcccagaccctcaaccaatcggagaacctcccgcagccccctcaggtgtgggatctcttacaatggcttcaggtggtggcgcaccagtggcagacaataacgaaggtgccgatggagtgggtagttcctcgggaaattggcattgcgattcccaatggctgggggacagagtcatcaccaccagcacccgaacctgggccctgcccacctacaacaatcacctctacaagcaaatctccaacagcacatctggaggatcttcaaatgacaacgcctacttcggctacagcaccccctgggggtattttgacttcaacagattccactgccacttctcaccacgtgactggcagcgactcatcaacaacaactggggattccggcctaagcgactcaacttcaagctcttcaacattcaggtcaaagaggttacggacaacaatggagtcaagaccatcgccaataaccttaccagcacggtccaggtcttcacggactcagactatcagctcccgtacgtgctcgggtcggctcacgagggctgcctcccgccgttcccagcggacgttttcatgattcctcagtacgggtatctgacgcttaatgatggaagccaggccgtgggtcgttcgtccttttactgcctggaatatttcccgtcgcaaatgctaagaacgggtaacaacttccagttcagctacgagtttgagaacgtacctttccatagcagctacgctcacagccaaagcctggaccgactaatgaatccactcatcgaccaatacttgtactatctctcaaagactattaacggttctggacagaatcaacaaacgctaaaattcagtgtggccggacccagcaacatggctgtccagggaagaaactacatacctggacccagctaccgacaacaacgtgtctcaaccactgtgactcaaaacaacaacagcgaatttgcttggcctggagcttcttcttgggctctcaatggacgtaatagcttgatgaatcctggacctgctatggccagccacaaagaaggagaggaccgtttctttcctttgtctggatctttaatttttggcaaacaaggaactggaagagacaacgtggatgcggacaaagtcatgataaccaacgaagaagaaattaaaactactaacccggtagcaacggagtcctatggacaagtggccacaaaccaccagagtgcccaagcacaggcgcagaccggctgggttcaaaaccaaggaatgcttccgggtatggtttggcaggacagagatgtgtacctgcaaggacccatttgggccaaaattcctcacacggacggcaactttcacccttctccgctgatgggagggtttggaatgaagcacccgcctcctcagatcctcatcaaaaacacacctgtacctgcggatcctccaacggccttcaacaaggacaagctgaactctttcatcacccagtattctactggccaagtcagcgtggagatcgagtgggagctgcagaaggaaaacagcaagcgctggaacccggagatccagtacacttccaactattacaagtctaataatgttgaatttgctgttaatactgaaggtgtatatagtgaaccccgccccattggcaccagatacctgactcgtaatctgtaa

SEQ ID NO: 9 - protein, 599 aa, Adeno-associated dependoparvovirus A
TAPGKKRPVEQSPQEPDSSAGIGKSGAQPAKKRLNFGQTGDTESVPDPQPIGEPPAAPSGVGSLTMASGGGAPVADNNEGADGVGSSSGNWHCDSQWLGDRVITTSTRTWALPTYNNHLYKQISNSTSGGSSNDNAYFGYSTPWGYFDFNRFHCHFSPRDWQRLINNNWGFRPKRLNFKLFNIQVKEVTDNNGVKTIANNLTSTVQVFTDSDYQLPYVLGSAHEGCLPPFPADVFMIPQYGYLTLNDGSQAVGRSSFYCLEYFPSQMLRTGNNFQFSYEFENVPFHSSYAHSQSLDRLMNPLIDQYLYYLSKTINGSGQNQQTLKFSVAGPSNMAVQGRNYIPGPSYRQQRVSTTVTQNNNSEFAWPGASSWALNGRNSLMNPGPAMASHKEGEDRFFPLSGSLIFGKQGTGRDNVDADKVMITNEEEIKTTNPVATESYGQVATNHQSAQAQAQTGWVQNQGILPGMVWQDRDVYLQGPIWAKIPHTDGNFHPSPLMGGFGMKHPPPQILIKNTPVPADPPTAFNKDKLNSFITQYSTGQVSVEIEWELQKENSKRWNPEIQYTSNYYKSNNVEFAVNTEGVYSEPRPIGTRYLTRNL

SEQ ID NO: 10 - protein, 599 aa, synthetic construct
TAPGKKRPVEQSPQEPDSSAGIGKSGAQPAKKRLNFGQTGDTESVPDPQPIGEPPAAPSGVGSLTMASGGGAPVADNNEGADGVGSSSGNWHCDSQWLGDRVITTSTRTWALPTYNNHLYKQISNSTSGGSSNDNAYFGYSTPWGYFDFNRFHCHFSPRDWQRLINNNWGFRPKRLNFKLFNIQVKEVTDNNGVKTIANNLTSTVQVFTDSDYQLPYVLGSAHEGCLPPFPADVFMIPQYGYLTLNDGSQAVGRSSFYCLEYFPSQMLRTGNNFQFSYEFENVPWHSSYAHSQSLDRLMNPLIDQYLYYLSKTINGSGQNQQTLKFSVAGPSNMAVQGRNYIPGPSYRQQRVSTTVTQNNNSEFAWPGASSWALNGRNSLMNPGPAMASHKEGEDRFFPLSGSLIFGKQGTGRDNVDADKVMITNEEEIKTTNPVATESYGQVATNHQSAQAQAQTGWVQNQGILPGMVWQDRDVYLQGPIWAKIPHTDGNFHPSPLMGGFGMKHPPPQILIKNTPVPADPPTAFNKDKLNSFITQYSTGQVSVEIEWELQKENSKRWNPEIQYTSNYYKSNNVEFAVNTEGVYSEPRPIGTRYLTRNL

SEQ ID NO: 11 - protein, 599 aa, synthetic construct
TAPGKKRPVEQSPQEPDSSAGIGKSGAQPAKKRLNFGQTGDTESVPDPQPIGEPPAAPSGVGSLTMASGGGAPVADNNEGADGVGSSSGNWHCDSQWLGDRVITTSTRTWALPTYNNHLYKQISNSTSGGSSNDNAYFGYSTPWGYFDFNRFHCHFSPRDWQRLINNNWGFRPKRLNFKLFNIQVKEVTDNNGVKTIANNLTSTVQVFTDSDYQLPYVLGSAHEGCLPPFPADVFMIPQYGYLTLNDGSQAVGRSSFYCLEYFPSQMLRTGNNFQFSYEFENVPWHSSYAHSQSLDRLMNPLIDQYLYFLSKTINGSGQNQQTLKFSVAGPSNMAVQGRNYIPGPSYRQQRVSTTVTQNNNSEFAWPGASSWALNGRNSLMNPGPAMASHKEGEDRFFPLSGSLIFGKQGTGRDNVDADKVMITNEEEIKTTNPVATESYGQVATNHQSAQAQAQTGWVQNQGILPGMVWQDRDVYLQGPIWAKIPHTDGNFHPSPLMGGFGMKHPPPQILIKNTPVPADPPTAFNKDKLNSFITQYSTGQVSVEIEWELQKENSKRWNPEIQYTSNYYKSNNVEFAVNTEGVYSEPRPIGTRYLTRNL

SEQ ID NO: 12 - protein, 599 aa, synthetic construct
TAPGKKRPVEQSPQEPDSSAGIGKSGAQPAKKRLNFGQTGDTESVPDPQPIGEPPAAPSGVGSLTMASGGGAPVADNNEGADGVGSSSGNWHCDSQWLGDRVITTSTRTWALPTYNNHLYKQISNSTSGGSSNDNAYFGYSTPWGYFDFNRFHCHFSPRDWQRLINNNWGFRPKRLNFKLFNIQVKEVTDNNGVKTIANNLTSTVQVFTDSDYQLPYVLGSAHEGCLPPFPADVFMIPQYGYLTLNDGSQAVGRSSFYCLEYFPSQMLRTGNNFQFSYEFENVPFHSSYAHSQSLDRLMNPLIDQYLYYLSKTINGSGQNQQTLKFSVAGPSNMAVQGRNYIPGPSYRQQRVSTTVTQNNNSEFAWPGASSWALNGRNSLMNPGPAMASHKEGEDRFFPLSGSLIFGKQGTGRDNVDADKVMITNEEEIKTTNPVATESYGQVATNHQSAQAQAQTGWVQNQGMLPGMVWQDRDVYLQGPIWAKIPHTDGNFHPSPLMGGFGMKHPPPQILIKNTPVPADPPTAFNKDKLNSFITQYSTGQVSVEIEWELQKENSKRWNPEIQYTSNYYKSNNVEFAVNTEGVYSEPRPIGTRYLTRNL

SEQ ID NO: 13 - DNA, 1800 bp, Adeno-associated dependoparvovirus A
  source 1..1800: mol_type = genomic DNA
acggctcctggaaagaagaggcctgtagagcagtctcctcaggaaccggactcctccgcgggtattggcaaatcgggtgcacagcccgctaaaaagagactcaatttcggtcagactggcgacacagagtcagtcccagaccctcaaccaatcggagaacctcccgcagccccctcaggtgtgggatctcttacaatggcttcaggtggtggcgcaccagtggcagacaataacgaaggtgccgatggagtgggtagttcctcgggaaattggcattgcgattcccaatggctgggggacagagtcatcaccaccagcacccgaacctgggccctgcccacctacaacaatcacctctacaagcaaatctccaacagcacatctggaggatcttcaaatgacaacgcctacttcggctacagcaccccctgggggtattttgacttcaacagattccactgccacttctcaccacgtgactggcagcgactcatcaacaacaactggggattccggcctaagcgactcaacttcaagctcttcaacattcaggtcaaagaggttacggacaacaatggagtcaagaccatcgccaataaccttaccagcacggtccaggtcttcacggactcagactatcagctcccgtacgtgctcgggtcggctcacgagggctgcctcccgccgttcccagcggacgttttcatgattcctcagtacgggtatctgacgcttaatgatggaagccaggccgtgggtcgttcgtccttttactgcctggaatatttcccgtcgcaaatgctaagaacgggtaacaacttccagttcagctacgagtttgagaacgtacctttccatagcagctacgctcacagccaaagcctggaccgactaatgaatccactcatcgaccaatacttgtactatctctcaaagactattaacggttctggacagaatcaacaaacgctaaaattcagtgtggccggacccagcaacatggctgtccagggaagaaactacatacctggacccagctaccgacaacaacgtgtctcaaccactgtgactcaaaacaacaacagcgaatttgcttggcctggagcttcttcttgggctctcaatggacgtaatagcttgatgaatcctggacctgctatggccagccacaaagaaggagaggaccgtttctttcctttgtctggatctttaatttttggcaaacaaggaactggaagagacaacgtggatgcggacaaagtcatgataaccaacgaagaagaaattaaaactactaacccggtagcaacggagtcctatggacaagtggccacaaaccaccagagtgcccaagcacaggcgcagaccggctgggttcaaaaccaaggaatacttccgggtatggtttggcaggacagagatgtgtacctgcaaggacccatttgggccaaaattcctcacacggacggcaactttcacccttctccgctgatgggagggtttggaatgaagcacccgcctcctcagatcctcatcaaaaacacacctgtacctgcggatcctccaacggccttcaacaaggacaagctgaactctttcatcacccagtattctactggccaagtcagcgtggagatcgagtgggagctgcagaaggaaaacagcaagcgctggaacccggagatccagtacacttccaactattacaagtctaataatgttgaatttgctgttaatactgaaggtgtatatagtgaaccccgccccattggcaccagatacctgactcgtaatctgtaa

SEQ ID NO: 14 - DNA, 1800 bp, synthetic construct
  source 1..1800: mol_type = other DNA
acggctcctggaaagaagaggcctgtagagcagtctcctcaggaaccggactcctccgcgggtattggcaaatcgggtgcacagcccgctaaaaagagactcaatttcggtcagactggcgacacagagtcagtcccagaccctcaaccaatcggagaacctcccgcagccccctcaggtgtgggatctcttacaatggcttcaggtggtggcgcaccagtggcagacaataacgaaggtgccgatggagtgggtagttcctcgggaaattggcattgcgattcccaatggctgggggacagagtcatcaccaccagcacccgaacctgggccctgcccacctacaacaatcacctctacaagcaaatctccaacagcacatctggaggatcttcaaatgacaacgcctacttcggctacagcaccccctgggggtattttgacttcaacagattccactgccacttctcaccacgtgactggcagcgactcatcaacaacaactggggattccggcctaagcgactcaacttcaagctcttcaacattcaggtcaaagaggttacggacaacaatggagtcaagaccatcgccaataaccttaccagcacggtccaggtcttcacggactcagactatcagctcccgtacgtgctcgggtcggctcacgagggctgcctcccgccgttcccagcggacgttttcatgattcctcagtacgggtatctgacgcttaatgatggaagccaggccgtgggtcgttcgtccttttactgcctggaatatttcccgtcgcaaatgctaagaacgggtaacaacttccagttcagctacgagtttgagaacgtaccttggcatagcagctacgctcacagccaaagcctggaccgactaatgaatccactcatcgaccaatacttgtactatctctcaaagactattaacggttctggacagaatcaacaaacgctaaaattcagtgtggccggacccagcaacatggctgtccagggaagaaactacatacctggacccagctaccgacaacaacgtgtctcaaccactgtgactcaaaacaacaacagcgaatttgcttggcctggagcttcttcttgggctctcaatggacgtaatagcttgatgaatcctggacctgctatggccagccacaaagaaggagaggaccgtttctttcctttgtctggatctttaatttttggcaaacaaggaactggaagagacaacgtggatgcggacaaagtcatgataaccaacgaagaagaaattaaaactactaacccggtagcaacggagtcctatggacaagtggccacaaaccaccagagtgcccaagcacaggcgcagaccggctgggttcaaaaccaaggaatacttccgggtatggtttggcaggacagagatgtgtacctgcaaggacccatttgggccaaaattcctcacacggacggcaactttcacccttctccgctgatgggagggtttggaatgaagcacccgcctcctcagatcctcatcaaaaacacacctgtacctgcggatcctccaacggccttcaacaaggacaagctgaactctttcatcacccagtattctactggccaagtcagcgtggagatcgagtgggagctgcagaaggaaaacagcaagcgctggaacccggagatccagtacacttccaactattacaagtctaataatgttgaatttgctgttaatactgaaggtgtatatagtgaaccccgccccattggcaccagatacctgactcgtaatctgtaa

SEQ ID NO: 15 - DNA, 1800 bp, synthetic construct
  source 1..1800: mol_type = other DNA
acggctcctggaaagaagaggcctgtagagcagtctcctcaggaaccggactcctccgcgggtattggcaaatcgggtgcacagcccgctaaaaagagactcaatttcggtcagactggcgacacagagtcagtcccagaccctcaaccaatcggagaacctcccgcagccccctcaggtgtgggatctcttacaatggcttcaggtggtggcgcaccagtggcagacaataacgaaggtgccgatggagtgggtagttcctcgggaaattggcattgcgattcccaatggctgggggacagagtcatcaccaccagcacccgaacctgggccctgcccacctacaacaatcacctctacaagcaaatctccaacagcacatctggaggatcttcaaatgacaacgcctacttcggctacagcaccccctgggggtattttgacttcaacagattccactgccacttctcaccacgtgactggcagcgactcatcaacaacaactggggattccggcctaagcgactcaacttcaagctcttcaacattcaggtcaaagaggttacggacaacaatggagtcaagaccatcgccaataaccttaccagcacggtccaggtcttcacggactcagactatcagctcccgtacgtgctcgggtcggctcacgagggctgcctcccgccgttcccagcggacgttttcatgattcctcagtacgggtatctgacgcttaatgatggaagccaggccgtgggtcgttcgtccttttactgcctggaatatttcccgtcgcaaatgctaagaacgggtaacaacttccagttcagctacgagtttgagaacgtaccttggcatagcagctacgctcacagccaaagcctggaccgactaatgaatccactcatcgaccaatacttgtactttctctcaaagactattaacggttctggacagaatcaacaaacgctaaaattcagtgtggccggacccagcaacatggctgtccagggaagaaactacatacctggacccagctaccgacaacaacgtgtctcaaccactgtgactcaaaacaacaacagcgaatttgcttggcctggagcttcttcttgggctctcaatggacgtaatagcttgatgaatcctggacctgctatggccagccacaaagaaggagaggaccgtttctttcctttgtctggatctttaatttttggcaaacaaggaactggaagagacaacgtggatgcggacaaagtcatgataaccaacgaagaagaaattaaaactactaacccggtagcaacggagtcctatggacaagtggccacaaaccaccagagtgcccaagcacaggcgcagaccggctgggttcaaaaccaaggaatacttccgggtatggtttggcaggacagagatgtgtacctgcaaggacccatttgggccaaaattcctcacacggacggcaactttcacccttctccgctgatgggagggtttggaatgaagcacccgcctcctcagatcctcatcaaaaacacacctgtacctgcggatcctccaacggccttcaacaaggacaagctgaactctttcatcacccagtattctactggccaagtcagcgtggagatcgagtgggagctgcagaaggaaaacagcaagcgctggaacccggagatccagtacacttccaactattacaagtctaataatgttgaatttgctgttaatactgaaggtgtatatagtgaaccccgccccattggcaccagatacctgactcgtaatctgtaa

SEQ ID NO: 16 - DNA, 1800 bp, synthetic construct
  source 1..1800: mol_type = other DNA
acggctcctggaaagaagaggcctgtagagcagtctcctcaggaaccggactcctccgcgggtattggcaaatcgggtgcacagcccgctaaaaagagactcaatttcggtcagactggcgacacagagtcagtcccagaccctcaaccaatcggagaacctcccgcagccccctcaggtgtgggatctcttacaatggcttcaggtggtggcgcaccagtggcagacaataacgaaggtgccgatggagtgggtagttcctcgggaaattggcattgcgattcccaatggctgggggacagagtcatcaccaccagcacccgaacctgggccctgcccacctacaacaatcacctctacaagcaaatctccaacagcacatctggaggatcttcaaatgacaacgcctacttcggctacagcaccccctgggggtattttgacttcaacagattccactgccacttctcaccacgtgactggcagcgactcatcaacaacaactggggattccggcctaagcgactcaacttcaagctcttcaacattcaggtcaaagaggttacggacaacaatggagtcaagaccatcgccaataaccttaccagcacggtccaggtcttcacggactcagactatcagctcccgtacgtgctcgggtcggctcacgagggctgcctcccgccgttcccagcggacgttttcatgattcctcagtacgggtatctgacgcttaatgatggaagccaggccgtgggtcgttcgtccttttactgcctggaatatttcccgtcgcaaatgctaagaacgggtaacaacttccagttcagctacgagtttgagaacgtacctttccatagcagctacgctcacagccaaagcctggaccgactaatgaatccactcatcgaccaatacttgtactatctctcaaagactattaacggttctggacagaatcaacaaacgctaaaattcagtgtggccggacccagcaacatggctgtccagggaagaaactacatacctggacccagctaccgacaacaacgtgtctcaaccactgtgactcaaaacaacaacagcgaatttgcttggcctggagcttcttcttgggctctcaatggacgtaatagcttgatgaatcctggacctgctatggccagccacaaagaaggagaggaccgtttctttcctttgtctggatctttaatttttggcaaacaaggaactggaagagacaacgtggatgcggacaaagtcatgataaccaacgaagaagaaattaaaactactaacccggtagcaacggagtcctatggacaagtggccacaaaccaccagagtgcccaagcacaggcgcagaccggctgggttcaaaaccaaggaatgcttccgggtatggtttggcaggacagagatgtgtacctgcaaggacccatttgggccaaaattcctcacacggacggcaactttcacccttctccgctgatgggagggtttggaatgaagcacccgcctcctcagatcctcatcaaaaacacacctgtacctgcggatcctccaacggccttcaacaaggacaagctgaactctttcatcacccagtattctactggccaagtcagcgtggagatcgagtgggagctgcagaaggaaaacagcaagcgctggaacccggagatccagtacacttccaactattacaagtctaataatgttgaatttgctgttaatactgaaggtgtatatagtgaaccccgccccattggcaccagatacctgactcgtaatctgtaa

SEQ ID NO: 17 - protein, 534 aa, Adeno-associated dependoparvovirus A
MASGGGAPVADNNEGADGVGSSSGNWHCDSQWLGDRVITTSTRTWALPTYNNHLYKQISNSTSGGSSNDNAYFGYSTPWGYFDFNRFHCHFSPRDWQRLINNNWGFRPKRLNFKLFNIQVKEVTDNNGVKTIANNLTSTVQVFTDSDYQLPYVLGSAHEGCLPPFPADVFMIPQYGYLTLNDGSQAVGRSSFYCLEYFPSQMLRTGNNFQFSYEFENVPFHSSYAHSQSLDRLMNPLIDQYLYYLSKTINGSGQNQQTLKFSVAGPSNMAVQGRNYIPGPSYRQQRVSTTVTQNNNSEFAWPGASSWALNGRNSLMNPGPAMASHKEGEDRFFPLSGSLIFGKQGTGRDNVDADKVMITNEEEIKTTNPVATESYGQVATNHQSAQAQAQTGWVQNQGILPGMVWQDRDVYLQGPIWAKIPHTDGNFHPSPLMGGFGMKHPPPQILIKNTPVPADPPTAFNKDKLNSFITQYSTGQVSVEIEWELQKENSKRWNPEIQYTSNYYKSNNVEFAVNTEGVYSEPRPIGTRYLTRNL

SEQ ID NO: 18 - protein, 534 aa, synthetic construct
MASGGGAPVADNNEGADGVGSSSGNWHCDSQWLGDRVITTSTRTWALPTYNNHLYKQISNSTSGGSSNDNAYFGYSTPWGYFDFNRFHCHFSPRDWQRLINNNWGFRPKRLNFKLFNIQVKEVTDNNGVKTIANNLTSTVQVFTDSDYQLPYVLGSAHEGCLPPFPADVFMIPQYGYLTLNDGSQAVGRSSFYCLEYFPSQMLRTGNNFQFSYEFENVPWHSSYAHSQSLDRLMNPLIDQYLYYLSKTINGSGQNQQTLKFSVAGPSNMAVQGRNYIPGPSYRQQRVSTTVTQNNNSEFAWPGASSWALNGRNSLMNPGPAMASHKEGEDRFFPLSGSLIFGKQGTGRDNVDADKVMITNEEEIKTTNPVATESYGQVATNHQSAQAQAQTGWVQNQGILPGMVWQDRDVYLQGPIWAKIPHTDGNFHPSPLMGGFGMKHPPPQILIKNTPVPADPPTAFNKDKLNSFITQYSTGQVSVEIEWELQKENSKRWNPEIQYTSNYYKSNNVEFAVNTEGVYSEPRPIGTRYLTRNL

SEQ ID NO: 19 - protein, 534 aa, synthetic construct
MASGGGAPVADNNEGADGVGSSSGNWHCDSQWLGDRVITTSTRTWALPTYNNHLYKQISNSTSGGSSNDNAYFGYSTPWGYFDFNRFHCHFSPRDWQRLINNNWGFRPKRLNFKLFNIQVKEVTDNNGVKTIANNLTSTVQVFTDSDYQLPYVLGSAHEGCLPPFPADVFMIPQYGYLTLNDGSQAVGRSSFYCLEYFPSQMLRTGNNFQFSYEFENVPWHSSYAHSQSLDRLMNPLIDQYLYFLSKTINGSGQNQQTLKFSVAGPSNMAVQGRNYIPGPSYRQQRVSTTVTQNNNSEFAWPGASSWALNGRNSLMNPGPAMASHKEGEDRFFPLSGSLIFGKQGTGRDNVDADKVMITNEEEIKTTNPVATESYGQVATNHQSAQAQAQTGWVQNQGILPGMVWQDRDVYLQGPIWAKIPHTDGNFHPSPLMGGFGMKHPPPQILIKNTPVPADPPTAFNKDKLNSFITQYSTGQVSVEIEWELQKENSKRWNPEIQYTSNYYKSNNVEFAVNTEGVYSEPRPIGTRYLTRNL

SEQ ID NO: 20 - protein, 534 aa, synthetic construct
MASGGGAPVADNNEGADGVGSSSGNWHCDSQWLGDRVITTSTRTWALPTYNNHLYKQISNSTSGGSSNDNAYFGYSTPWGYFDFNRFHCHFSPRDWQRLINNNWGFRPKRLNFKLFNIQVKEVTDNNGVKTIANNLTSTVQVFTDSDYQLPYVLGSAHEGCLPPFPADVFMIPQYGYLTLNDGSQAVGRSSFYCLEYFPSQMLRTGNNFQFSYEFENVPFHSSYAHSQSLDRLMNPLIDQYLYYLSKTINGSGQNQQTLKFSVAGPSNMAVQGRNYIPGPSYRQQRVSTTVTQNNNSEFAWPGASSWALNGRNSLMNPGPAMASHKEGEDRFFPLSGSLIFGKQGTGRDNVDADKVMITNEEEIKTTNPVATESYGQVATNHQSAQAQAQTGWVQNQGMLPGMVWQDRDVYLQGPIWAKIPHTDGNFHPSPLMGGFGMKHPPPQILIKNTPVPADPPTAFNKDKLNSFITQYSTGQVSVEIEWELQKENSKRWNPEIQYTSNYYKSNNVEFAVNTEGVYSEPRPIGTRYLTRNL

SEQ ID NO: 21 - DNA, 1605 bp, Adeno-associated dependoparvovirus A
  source 1..1605: mol_type = genomic DNA
atggcttcaggtggtggcgcaccagtggcagacaataacgaaggtgccgatggagtgggtagttcctcgggaaattggcattgcgattcccaatggctgggggacagagtcatcaccaccagcacccgaacctgggccctgcccacctacaacaatcacctctacaagcaaatctccaacagcacatctggaggatcttcaaatgacaacgcctacttcggctacagcaccccctgggggtattttgacttcaacagattccactgccacttctcaccacgtgactggcagcgactcatcaacaacaactggggattccggcctaagcgactcaacttcaagctcttcaacattcaggtcaaagaggttacggacaacaatggagtcaagaccatcgccaataaccttaccagcacggtccaggtcttcacggactcagactatcagctcccgtacgtgctcgggtcggctcacgagggctgcctcccgccgttcccagcggacgttttcatgattcctcagtacgggtatctgacgcttaatgatggaagccaggccgtgggtcgttcgtccttttactgcctggaatatttcccgtcgcaaatgctaagaacgggtaacaacttccagttcagctacgagtttgagaacgtacctttccatagcagctacgctcacagccaaagcctggaccgactaatgaatccactcatcgaccaatacttgtactatctctcaaagactattaacggttctggacagaatcaacaaacgctaaaattcagtgtggccggacccagcaacatggctgtccagggaagaaactacatacctggacccagctaccgacaacaacgtgtctcaaccactgtgactcaaaacaacaacagcgaatttgcttggcctggagcttcttcttgggctctcaatggacgtaatagcttgatgaatcctggacctgctatggccagccacaaagaaggagaggaccgtttctttcctttgtctggatctttaatttttggcaaacaaggaactggaagagacaacgtggatgcggacaaagtcatgataaccaacgaagaagaaattaaaactactaacccggtagcaacggagtcctatggacaagtggccacaaaccaccagagtgcccaagcacaggcgcagaccggctgggttcaaaaccaaggaatacttccgggtatggtttggcaggacagagatgtgtacctgcaaggacccatttgggccaaaattcctcacacggacggcaactttcacccttctccgctgatgggagggtttggaatgaagcacccgcctcctcagatcctcatcaaaaacacacctgtacctgcggatcctccaacggccttcaacaaggacaagctgaactctttcatcacccagtattctactggccaagtcagcgtggagatcgagtgggagctgcagaaggaaaacagcaagcgctggaacccggagatccagtacacttccaactattacaagtctaataatgttgaatttgctgttaatactgaaggtgtatatagtgaaccccgccccattggcaccagatacctgactcgtaatctgtaa

SEQ ID NO: 22 - DNA, 1605 bp, synthetic construct
  source 1..1605: mol_type = other DNA
atggcttcaggtggtggcgcaccagtggcagacaataacgaaggtgccgatggagtgggtagttcctcgggaaattggcattgcgattcccaatggctgggggacagagtcatcaccaccagcacccgaacctgggccctgcccacctacaacaatcacctctacaagcaaatctccaacagcacatctggaggatcttcaaatgacaacgcctacttcggctacagcaccccctgggggtattttgacttcaacagattccactgccacttctcaccacgtgactggcagcgactcatcaacaacaactggggattccggcctaagcgactcaacttcaagctcttcaacattcaggtcaaagaggttacggacaacaatggagtcaagaccatcgccaataaccttaccagcacggtccaggtcttcacggactcagactatcagctcccgtacgtgctcgggtcggctcacgagggctgcctcccgccgttcccagcggacgttttcatgattcctcagtacgggtatctgacgcttaatgatggaagccaggccgtgggtcgttcgtccttttactgcctggaatatttcccgtcgcaaatgctaagaacgggtaacaacttccagttcagctacgagtttgagaacgtaccttggcatagcagctacgctcacagccaaagcctggaccgactaatgaatccactcatcgaccaatacttgtactatctctcaaagactattaacggttctggacagaatcaacaaacgctaaaattcagtgtggccggacccagcaacatggctgtccagggaagaaactacatacctggacccagctaccgacaacaacgtgtctcaaccactgtgactcaaaacaacaacagcgaatttgcttggcctggagcttcttcttgggctctcaatggacgtaatagcttgatgaatcctggacctgctatggccagccacaaagaaggagaggaccgtttctttcctttgtctggatctttaatttttggcaaacaaggaactggaagagacaacgtggatgcggacaaagtcatgataaccaacgaagaagaaattaaaactactaacccggtagcaacggagtcctatggacaagtggccacaaaccaccagagtgcccaagcacaggcgcagaccggctgggttcaaaaccaaggaatacttccgggtatggtttggcaggacagagatgtgtacctgcaaggacccatttgggccaaaattcctcacacggacggcaactttcacccttctccgctgatgggagggtttggaatgaagcacccgcctcctcagatcctcatcaaaaacacacctgtacctgcggatcctccaacggccttcaacaaggacaagctgaactctttcatcacccagtattctactggccaagtcagcgtggagatcgagtgggagctgcagaaggaaaacagcaagcgctggaacccggagatccagtacacttccaactattacaagtctaataatgttgaatttgctgttaatactgaaggtgtatatagtgaaccccgccccattggcaccagatacctgactcgtaatctgtaa

SEQ ID NO: 23 - DNA, 1605 bp, synthetic construct
  source 1..1605: mol_type = other DNA
atggcttcaggtggtggcgcaccagtggcagacaataacgaaggtgccgatggagtgggtagttcctcgggaaattggcattgcgattcccaatggctgggggacagagtcatcaccaccagcacccgaacctgggccctgcccacctacaacaatcacctctacaagcaaatctccaacagcacatctggaggatcttcaaatgacaacgcctacttcggctacagcaccccctgggggtattttgacttcaacagattccactgccacttctcaccacgtgactggcagcgactcatcaacaacaactggggattccggcctaagcgactcaacttcaagctcttcaacattcaggtcaaagaggttacggacaacaatggagtcaagaccatcgccaataaccttaccagcacggtccaggtcttcacggactcagactatcagctcccgtacgtgctcgggtcggctcacgagggctgcctcccgccgttcccagcggacgttttcatgattcctcagtacgggtatctgacgcttaatgatggaagccaggccgtgggtcgttcgtccttttactgcctggaatatttcccgtcgcaaatgctaagaacgggtaacaacttccagttcagctacgagtttgagaacgtaccttggcatagcagctacgctcacagccaaagcctggaccgactaatgaatccactcatcgaccaatacttgtactttctctcaaagactattaacggttctggacagaatcaacaaacgctaaaattcagtgtggccggacccagcaacatggctgtccagggaagaaactacatacctggacccagctaccgacaacaacgtgtctcaaccactgtgactcaaaacaacaacagcgaatttgcttggcctggagcttcttcttgggctctcaatggacgtaatagcttgatgaatcctggacctgctatggccagccacaaagaaggagaggaccgtttctttcctttgtctggatctttaatttttggcaaacaaggaactggaagagacaacgtggatgcggacaaagtcatgataaccaacgaagaagaaattaaaactactaacccggtagcaacggagtcctatggacaagtggccacaaaccaccagagtgcccaagcacaggcgcagaccggctgggttcaaaaccaaggaatacttccgggtatggtttggcaggacagagatgtgtacctgcaaggacccatttgggccaaaattcctcacacggacggcaactttcacccttctccgctgatgggagggtttggaatgaagcacccgcctcctcagatcctcatcaaaaacacacctgtacctgcggatcctccaacggccttcaacaaggacaagctgaactctttcatcacccagtattctactggccaagtcagcgtggagatcgagtgggagctgcagaaggaaaacagcaagcgctggaacccggagatccagtacacttccaactattacaagtctaataatgttgaatttgctgttaatactgaaggtgtatatagtgaaccccgccccattggcaccagatacctgactcgtaatctgtaa

SEQ ID NO: 24 - DNA, 1605 bp, synthetic construct
  source 1..1605: mol_type = other DNA
atggcttcaggtggtggcgcaccagtggcagacaataacgaaggtgccgatggagtgggtagttcctcgggaaattggcattgcgattcccaatggctgggggacagagtcatcaccaccagcacccgaacctgggccctgcccacctacaacaatcacctctacaagcaaatctccaacagcacatctggaggatcttcaaatgacaacgcctacttcggctacagcaccccctgggggtattttgacttcaacagattccactgccacttctcaccacgtgactggcagcgactcatcaacaacaactggggattccggcctaagcgactcaacttcaagctcttcaacattcaggtcaaagaggttacggacaacaatggagtcaagaccatcgccaataaccttaccagcacggtccaggtcttcacggactcagactatcagctcccgtacgtgctcgggtcggctcacgagggctgcctcccgccgttcccagcggacgttttcatgattcctcagtacgggtatctgacgcttaatgatggaagccaggccgtgggtcgttcgtccttttactgcctggaatatttcccgtcgcaaatgctaagaacgggtaacaacttccagttcagctacgagtttgagaacgtacctttccatagcagctacgctcacagccaaagcctggaccgactaatgaatccactcatcgaccaatacttgtactatctctcaaagactattaacggttctggacagaatcaacaaacgctaaaattcagtgtggccggacccagcaacatggctgtccagggaagaaactacatacctggacccagctaccgacaacaacgtgtctcaaccactgtgactcaaaacaacaacagcgaatttgcttggcctggagcttcttcttgggctctcaatggacgtaatagcttgatgaatcctggacctgctatggccagccacaaagaaggagaggaccgtttctttcctttgtctggatctttaatttttggcaaacaaggaactggaagagacaacgtggatgcggacaaagtcatgataaccaacgaagaagaaattaaaactactaacccggtagcaacggagtcctatggacaagtggccacaaaccaccagagtgcccaagcacaggcgcagaccggctgggttcaaaaccaaggaatgcttccgggtatggtttggcaggacagagatgtgtacctgcaaggacccatttgggccaaaattcctcacacggacggcaactttcacccttctccgctgatgggagggtttggaatgaagcacccgcctcctcagatcctcatcaaaaacacacctgtacctgcggatcctccaacggccttcaacaaggacaagctgaactctttcatcacccagtattctactggccaagtcagcgtggagatcgagtgggagctgcagaaggaaaacagcaagcgctggaacccggagatccagtacacttccaactattacaagtctaataatgttgaatttgctgttaatactgaaggtgtatatagtgaaccccgccccattggcaccagatacctgactcgtaatctgtaa